European Patent Specification EP 3 727 435 B1, published February 18, 2026. Title: BIVALENT NUCLEIC ACID LIGANDS AND USES THEREFOR. Applicant: Carnegie Mellon University. The sequence listing filed with the application follows.

SEQUENCE LISTING (1 sequence)

SEQ ID NO: 1 - RNA, 22 nt, Homo sapiens
cgccagcgcagcagcgcaggcg